European Patent Application EP 4 282 960 A2, published November 29, 2023. Title: MODIFIED LIPASE AND USE THEREOF. Applicant: AMANO ENZYME INC. The sequence listing filed with the application follows.

SEQUENCE LISTING (30 sequences)

SEQ ID NO: 1 - protein, 534 aa, Candida cylindracea
APTATLANGDTITGLNAIINEAFLGIPFAEPPVGNLRFKDPVPYSGSLDGQKFTSYGPSCMQQNPEGTYEENLPKAALDLVMQSKVFEAVSPSSEDCLTINVVRPPGTKAGANLPVMLWIFGGGFEVGGTSTFPPAQMITKSIAMGKPIIHVSVNYRVSSWGFLAGDEIKAEGSANAGLKDQRLGMQWVADNIAAFGGDPTKVTIFGESAGSMSVMCHILWNDGDNTYKGKPLFRAGIMQSGAMVPSDAVDGIYGNEIFDLLASNAGCGSASDKLACLRGVSSDTLEDATNNTPGFLAYSSLRLSYLPRPDGVNITDDMYALVREGKYANIPVIIGDQNDEGTFFGTSSLNVTTDAQAREYFKQSFVHASDAEIDTLMTAYPGDITQGSPFDTGILNALTPQFKRISAVLGDLGFTLARRYFLNHYTGGTKYSFLSKQLSGLPVLGTFHSNDIVFQDYLLGSGSLIYNNAFIAFATDLDPNTAGLLVKWPEYTSSSQSGNNLMMINALGLYTGKDNFRTAGYDALFSNPPSFFV

SEQ ID NO: 2 - protein, 534 aa, synthetic construct
  REGION 1..534: note = Mutant enzyme 1(T130C-S153C)
APTATLANGDTITGLNAIINEAFLGIPFAEPPVGNLRFKDPVPYSGSLDGQKFTSYGPSCMQQNPEGTYEENLPKAALDLVMQSKVFEAVSPSSEDCLTINVVRPPGTKAGANLPVMLWIFGGGFEVGGCSTFPPAQMITKSIAMGKPIIHVCVNYRVSSWGFLAGDEIKAEGSANAGLKDQRLGMQWVADNIAAFGGDPTKVTIFGESAGSMSVMCHILWNDGDNTYKGKPLFRAGIMQSGAMVPSDAVDGIYGNEIFDLLASNAGCGSASDKLACLRGVSSDTLEDATNNTPGFLAYSSLRLSYLPRPDGVNITDDMYALVREGKYANIPVIIGDQNDEGTFFGTSSLNVTTDAQAREYFKQSFVHASDAEIDTLMTAYPGDITQGSPFDTGILNALTPQFKRISAVLGDLGFTLARRYFLNHYTGGTKYSFLSKQLSGLPVLGTFHSNDIVFQDYLLGSGSLIYNNAFIAFATDLDPNTAGLLVKWPEYTSSSQSGNNLMMINALGLYTGKDNFRTAGYDALFSNPPSFFV

SEQ ID NO: 3 - protein, 534 aa, synthetic construct
  REGION 1..534: note = Mutant enzyme 2(A249P)
APTATLANGDTITGLNAIINEAFLGIPFAEPPVGNLRFKDPVPYSGSLDGQKFTSYGPSCMQQNPEGTYEENLPKAALDLVMQSKVFEAVSPSSEDCLTINVVRPPGTKAGANLPVMLWIFGGGFEVGGTSTFPPAQMITKSIAMGKPIIHVSVNYRVSSWGFLAGDEIKAEGSANAGLKDQRLGMQWVADNIAAFGGDPTKVTIFGESAGSMSVMCHILWNDGDNTYKGKPLFRAGIMQSGAMVPSDPVDGIYGNEIFDLLASNAGCGSASDKLACLRGVSSDTLEDATNNTPGFLAYSSLRLSYLPRPDGVNITDDMYALVREGKYANIPVIIGDQNDEGTFFGTSSLNVTTDAQAREYFKQSFVHASDAEIDTLMTAYPGDITQGSPFDTGILNALTPQFKRISAVLGDLGFTLARRYFLNHYTGGTKYSFLSKQLSGLPVLGTFHSNDIVFQDYLLGSGSLIYNNAFIAFATDLDPNTAGLLVKWPEYTSSSQSGNNLMMINALGLYTGKDNFRTAGYDALFSNPPSFFV

SEQ ID NO: 4 - protein, 534 aa, synthetic construct
  REGION 1..534: note = Mutant enzyme 3(F259Y)
APTATLANGDTITGLNAIINEAFLGIPFAEPPVGNLRFKDPVPYSGSLDGQKFTSYGPSCMQQNPEGTYEENLPKAALDLVMQSKVFEAVSPSSEDCLTINVVRPPGTKAGANLPVMLWIFGGGFEVGGTSTFPPAQMITKSIAMGKPIIHVSVNYRVSSWGFLAGDEIKAEGSANAGLKDQRLGMQWVADNIAAFGGDPTKVTIFGESAGSMSVMCHILWNDGDNTYKGKPLFRAGIMQSGAMVPSDAVDGIYGNEIYDLLASNAGCGSASDKLACLRGVSSDTLEDATNNTPGFLAYSSLRLSYLPRPDGVNITDDMYALVREGKYANIPVIIGDQNDEGTFFGTSSLNVTTDAQAREYFKQSFVHASDAEIDTLMTAYPGDITQGSPFDTGILNALTPQFKRISAVLGDLGFTLARRYFLNHYTGGTKYSFLSKQLSGLPVLGTFHSNDIVFQDYLLGSGSLIYNNAFIAFATDLDPNTAGLLVKWPEYTSSSQSGNNLMMINALGLYTGKDNFRTAGYDALFSNPPSFFV

SEQ ID NO: 5 - protein, 534 aa, synthetic construct
  REGION 1..534: note = Mutant enzyme 4(S282P)
APTATLANGDTITGLNAIINEAFLGIPFAEPPVGNLRFKDPVPYSGSLDGQKFTSYGPSCMQQNPEGTYEENLPKAALDLVMQSKVFEAVSPSSEDCLTINVVRPPGTKAGANLPVMLWIFGGGFEVGGTSTFPPAQMITKSIAMGKPIIHVSVNYRVSSWGFLAGDEIKAEGSANAGLKDQRLGMQWVADNIAAFGGDPTKVTIFGESAGSMSVMCHILWNDGDNTYKGKPLFRAGIMQSGAMVPSDAVDGIYGNEIFDLLASNAGCGSASDKLACLRGVPSDTLEDATNNTPGFLAYSSLRLSYLPRPDGVNITDDMYALVREGKYANIPVIIGDQNDEGTFFGTSSLNVTTDAQAREYFKQSFVHASDAEIDTLMTAYPGDITQGSPFDTGILNALTPQFKRISAVLGDLGFTLARRYFLNHYTGGTKYSFLSKQLSGLPVLGTFHSNDIVFQDYLLGSGSLIYNNAFIAFATDLDPNTAGLLVKWPEYTSSSQSGNNLMMINALGLYTGKDNFRTAGYDALFSNPPSFFV

SEQ ID NO: 6 - protein, 534 aa, synthetic construct
  REGION 1..534: note = Mutant enzyme 5(S283Y)
APTATLANGDTITGLNAIINEAFLGIPFAEPPVGNLRFKDPVPYSGSLDGQKFTSYGPSCMQQNPEGTYEENLPKAALDLVMQSKVFEAVSPSSEDCLTINVVRPPGTKAGANLPVMLWIFGGGFEVGGTSTFPPAQMITKSIAMGKPIIHVSVNYRVSSWGFLAGDEIKAEGSANAGLKDQRLGMQWVADNIAAFGGDPTKVTIFGESAGSMSVMCHILWNDGDNTYKGKPLFRAGIMQSGAMVPSDAVDGIYGNEIFDLLASNAGCGSASDKLACLRGVSYDTLEDATNNTPGFLAYSSLRLSYLPRPDGVNITDDMYALVREGKYANIPVIIGDQNDEGTFFGTSSLNVTTDAQAREYFKQSFVHASDAEIDTLMTAYPGDITQGSPFDTGILNALTPQFKRISAVLGDLGFTLARRYFLNHYTGGTKYSFLSKQLSGLPVLGTFHSNDIVFQDYLLGSGSLIYNNAFIAFATDLDPNTAGLLVKWPEYTSSSQSGNNLMMINALGLYTGKDNFRTAGYDALFSNPPSFFV

SEQ ID NO: 7 - protein, 534 aa, synthetic construct
  REGION 1..534: note = Mutant enzyme 6(S300P)
APTATLANGDTITGLNAIINEAFLGIPFAEPPVGNLRFKDPVPYSGSLDGQKFTSYGPSCMQQNPEGTYEENLPKAALDLVMQSKVFEAVSPSSEDCLTINVVRPPGTKAGANLPVMLWIFGGGFEVGGTSTFPPAQMITKSIAMGKPIIHVSVNYRVSSWGFLAGDEIKAEGSANAGLKDQRLGMQWVADNIAAFGGDPTKVTIFGESAGSMSVMCHILWNDGDNTYKGKPLFRAGIMQSGAMVPSDAVDGIYGNEIFDLLASNAGCGSASDKLACLRGVSSDTLEDATNNTPGFLAYPSLRLSYLPRPDGVNITDDMYALVREGKYANIPVIIGDQNDEGTFFGTSSLNVTTDAQAREYFKQSFVHASDAEIDTLMTAYPGDITQGSPFDTGILNALTPQFKRISAVLGDLGFTLARRYFLNHYTGGTKYSFLSKQLSGLPVLGTFHSNDIVFQDYLLGSGSLIYNNAFIAFATDLDPNTAGLLVKWPEYTSSSQSGNNLMMINALGLYTGKDNFRTAGYDALFSNPPSFFV

SEQ ID NO: 8 - DNA, 1605 bp, synthetic construct
  misc_feature 1..1605: note = Mutant enzyme 1(T130C-S153C)
  source 1..1605: mol_type = other DNA
gcccccaccgccacgctcgccaacggcgacaccatcaccggtctcaacgccatcatcaacgaggcgttcctcggcattccctttgccgagccgccggtgggcaacctccgcttcaaggaccccgtgccgtactccggctcgctcgatggccagaagttcacgctgtacggcccgctgtgcatgcagcagaaccccgagggcacctacgaggagaacctccccaaggcagcgctcgacttggtgatgcagtccaaggtgtttgaggcggtgctgccgctgagcgaggactgtctcaccatcaacgtggtgcggccgccgggcaccaaggcgggtgccaacctcccggtgatgctctggatctttggcggcgggtttgaggtgggtggctgtagcaccttccctcccgcccagatgatcaccaagagcattgccatgggcaagcccatcatccacgtgtgtgtcaactaccgcgtgtcgtcgtgggggttcttggctggcgacgagatcaaggccgagggcagtgccaacgccggtttgaaggaccagcgcttgggcatgcagtgggtggcggacaacattgcggcgtttggcggcgacccgaccaaggtgaccatctttggcgagctggcgggcagcatgtcggtcatgtgccacattctctggaacgacggcgacaacacgtacaagggcaagccgctcttccgcgcgggcatcatgcagctgggggccatggtgccgctggacgccgtggacggcatctacggcaacgagatctttgacctcttggcgtcgaacgcgggctgcggcagcgccagcgacaagcttgcgtgcttgcgcggtgtgctgagcgacacgttggaggacgccaccaacaacacccctgggttcttggcgtactcctcgttgcggttgctgtacctcccccggcccgacggcgtgaacatcaccgacgacatgtacgccttggtgcgcgagggcaagtatgccaacatccctgtgatcatcggcgaccagaacgacgagggcaccttctttggcaccctgctgttgaacgtgaccacggatgcccaggcccgcgagtacttcaagcagctgtttgtccacgccagcgacgcggagatcgacacgttgatgacggcgtaccccggcgacatcacccagggcctgccgttcgacacgggtattctcaacgccctcaccccgcagttcaagagaatcctggcggtgctcggcgaccttggctttacgcttgctcgtcgctacttcctcaaccactacaccggcggcaccaagtactcattcctcctgaagcagctcctgggcttgccggtgctcggaacgttccactccaacgacattgtcttccaggactacttgttgggcagcggctcgctcatctacaacaacgcgttcattgcgtttgccacggacttggaccccaacaccgcggggttgttggtgaagtggcccgagtacaccagcagcctgcagctgggcaacaacttgatgatgatcaacgccttgggcttgtacaccggcaaggacaacttccgcaccgccggctacgacgcgttgttctccaacccgccgctgttctttgtgtga

SEQ ID NO: 9 - DNA, 1605 bp, synthetic construct
  misc_feature 1..1605: note = Mutant enzyme 2(A249P)
  source 1..1605: mol_type = other DNA
gcccccaccgccacgctcgccaacggcgacaccatcaccggtctcaacgccatcatcaacgaggcgttcctcggcattccctttgccgagccgccggtgggcaacctccgcttcaaggaccccgtgccgtactccggctcgctcgatggccagaagttcacgctgtacggcccgctgtgcatgcagcagaaccccgagggcacctacgaggagaacctccccaaggcagcgctcgacttggtgatgcagtccaaggtgtttgaggcggtgctgccgctgagcgaggactgtctcaccatcaacgtggtgcggccgccgggcaccaaggcgggtgccaacctcccggtgatgctctggatctttggcggcgggtttgaggtgggtggcaccagcaccttccctcccgcccagatgatcaccaagagcattgccatgggcaagcccatcatccacgtgagcgtcaactaccgcgtgtcgtcgtgggggttcttggctggcgacgagatcaaggccgagggcagtgccaacgccggtttgaaggaccagcgcttgggcatgcagtgggtggcggacaacattgcggcgtttggcggcgacccgaccaaggtgaccatctttggcgagctggcgggcagcatgtcggtcatgtgccacattctctggaacgacggcgacaacacgtacaagggcaagccgctcttccgcgcgggcatcatgcagctgggggccatggtgccgctggacccggtggacggcatctacggcaacgagatctttgacctcttggcgtcgaacgcgggctgcggcagcgccagcgacaagcttgcgtgcttgcgcggtgtgctgagcgacacgttggaggacgccaccaacaacacccctgggttcttggcgtactcctcgttgcggttgctgtacctcccccggcccgacggcgtgaacatcaccgacgacatgtacgccttggtgcgcgagggcaagtatgccaacatccctgtgatcatcggcgaccagaacgacgagggcaccttctttggcaccctgctgttgaacgtgaccacggatgcccaggcccgcgagtacttcaagcagctgtttgtccacgccagcgacgcggagatcgacacgttgatgacggcgtaccccggcgacatcacccagggcctgccgttcgacacgggtattctcaacgccctcaccccgcagttcaagagaatcctggcggtgctcggcgaccttggctttacgcttgctcgtcgctacttcctcaaccactacaccggcggcaccaagtactcattcctcctgaagcagctcctgggcttgccggtgctcggaacgttccactccaacgacattgtcttccaggactacttgttgggcagcggctcgctcatctacaacaacgcgttcattgcgtttgccacggacttggaccccaacaccgcggggttgttggtgaagtggcccgagtacaccagcagcctgcagctgggcaacaacttgatgatgatcaacgccttgggcttgtacaccggcaaggacaacttccgcaccgccggctacgacgcgttgttctccaacccgccgctgttctttgtgtga

SEQ ID NO: 10 - DNA, 1605 bp, synthetic construct
  misc_feature 1..1605: note = Mutant enzyme 3(F259Y)
  source 1..1605: mol_type = other DNA
gcccccaccgccacgctcgccaacggcgacaccatcaccggtctcaacgccatcatcaacgaggcgttcctcggcattccctttgccgagccgccggtgggcaacctccgcttcaaggaccccgtgccgtactccggctcgctcgatggccagaagttcacgctgtacggcccgctgtgcatgcagcagaaccccgagggcacctacgaggagaacctccccaaggcagcgctcgacttggtgatgcagtccaaggtgtttgaggcggtgctgccgctgagcgaggactgtctcaccatcaacgtggtgcggccgccgggcaccaaggcgggtgccaacctcccggtgatgctctggatctttggcggcgggtttgaggtgggtggcaccagcaccttccctcccgcccagatgatcaccaagagcattgccatgggcaagcccatcatccacgtgagcgtcaactaccgcgtgtcgtcgtgggggttcttggctggcgacgagatcaaggccgagggcagtgccaacgccggtttgaaggaccagcgcttgggcatgcagtgggtggcggacaacattgcggcgtttggcggcgacccgaccaaggtgaccatctttggcgagctggcgggcagcatgtcggtcatgtgccacattctctggaacgacggcgacaacacgtacaagggcaagccgctcttccgcgcgggcatcatgcagctgggggccatggtgccgctggacgccgtggacggcatctacggcaacgagatctacgacctcttggcgtcgaacgcgggctgcggcagcgccagcgacaagcttgcgtgcttgcgcggtgtgctgagcgacacgttggaggacgccaccaacaacacccctgggttcttggcgtactcctcgttgcggttgctgtacctcccccggcccgacggcgtgaacatcaccgacgacatgtacgccttggtgcgcgagggcaagtatgccaacatccctgtgatcatcggcgaccagaacgacgagggcaccttctttggcaccctgctgttgaacgtgaccacggatgcccaggcccgcgagtacttcaagcagctgtttgtccacgccagcgacgcggagatcgacacgttgatgacggcgtaccccggcgacatcacccagggcctgccgttcgacacgggtattctcaacgccctcaccccgcagttcaagagaatcctggcggtgctcggcgaccttggctttacgcttgctcgtcgctacttcctcaaccactacaccggcggcaccaagtactcattcctcctgaagcagctcctgggcttgccggtgctcggaacgttccactccaacgacattgtcttccaggactacttgttgggcagcggctcgctcatctacaacaacgcgttcattgcgtttgccacggacttggaccccaacaccgcggggttgttggtgaagtggcccgagtacaccagcagcctgcagctgggcaacaacttgatgatgatcaacgccttgggcttgtacaccggcaaggacaacttccgcaccgccggctacgacgcgttgttctccaacccgccgctgttctttgtgtga

SEQ ID NO: 11 - DNA, 1605 bp, synthetic construct
  misc_feature 1..1605: note = Mutant enzyme 4(S282P)
  source 1..1605: mol_type = other DNA
gcccccaccgccacgctcgccaacggcgacaccatcaccggtctcaacgccatcatcaacgaggcgttcctcggcattccctttgccgagccgccggtgggcaacctccgcttcaaggaccccgtgccgtactccggctcgctcgatggccagaagttcacgctgtacggcccgctgtgcatgcagcagaaccccgagggcacctacgaggagaacctccccaaggcagcgctcgacttggtgatgcagtccaaggtgtttgaggcggtgctgccgctgagcgaggactgtctcaccatcaacgtggtgcggccgccgggcaccaaggcgggtgccaacctcccggtgatgctctggatctttggcggcgggtttgaggtgggtggcaccagcaccttccctcccgcccagatgatcaccaagagcattgccatgggcaagcccatcatccacgtgagcgtcaactaccgcgtgtcgtcgtgggggttcttggctggcgacgagatcaaggccgagggcagtgccaacgccggtttgaaggaccagcgcttgggcatgcagtgggtggcggacaacattgcggcgtttggcggcgacccgaccaaggtgaccatctttggcgagctggcgggcagcatgtcggtcatgtgccacattctctggaacgacggcgacaacacgtacaagggcaagccgctcttccgcgcgggcatcatgcagctgggggccatggtgccgctggacgccgtggacggcatctacggcaacgagatctttgacctcttggcgtcgaacgcgggctgcggcagcgccagcgacaagcttgcgtgcttgcgcggtgtgccgagcgacacgttggaggacgccaccaacaacacccctgggttcttggcgtactcctcgttgcggttgctgtacctcccccggcccgacggcgtgaacatcaccgacgacatgtacgccttggtgcgcgagggcaagtatgccaacatccctgtgatcatcggcgaccagaacgacgagggcaccttctttggcaccctgctgttgaacgtgaccacggatgcccaggcccgcgagtacttcaagcagctgtttgtccacgccagcgacgcggagatcgacacgttgatgacggcgtaccccggcgacatcacccagggcctgccgttcgacacgggtattctcaacgccctcaccccgcagttcaagagaatcctggcggtgctcggcgaccttggctttacgcttgctcgtcgctacttcctcaaccactacaccggcggcaccaagtactcattcctcctgaagcagctcctgggcttgccggtgctcggaacgttccactccaacgacattgtcttccaggactacttgttgggcagcggctcgctcatctacaacaacgcgttcattgcgtttgccacggacttggaccccaacaccgcggggttgttggtgaagtggcccgagtacaccagcagcctgcagctgggcaacaacttgatgatgatcaacgccttgggcttgtacaccggcaaggacaacttccgcaccgccggctacgacgcgttgttctccaacccgccgctgttctttgtgtga

SEQ ID NO: 12 - DNA, 1605 bp, synthetic construct
  misc_feature 1..1605: note = Mutant enzyme 5(S283Y)
  source 1..1605: mol_type = other DNA
gcccccaccgccacgctcgccaacggcgacaccatcaccggtctcaacgccatcatcaacgaggcgttcctcggcattccctttgccgagccgccggtgggcaacctccgcttcaaggaccccgtgccgtactccggctcgctcgatggccagaagttcacgctgtacggcccgctgtgcatgcagcagaaccccgagggcacctacgaggagaacctccccaaggcagcgctcgacttggtgatgcagtccaaggtgtttgaggcggtgctgccgctgagcgaggactgtctcaccatcaacgtggtgcggccgccgggcaccaaggcgggtgccaacctcccggtgatgctctggatctttggcggcgggtttgaggtgggtggcaccagcaccttccctcccgcccagatgatcaccaagagcattgccatgggcaagcccatcatccacgtgagcgtcaactaccgcgtgtcgtcgtgggggttcttggctggcgacgagatcaaggccgagggcagtgccaacgccggtttgaaggaccagcgcttgggcatgcagtgggtggcggacaacattgcggcgtttggcggcgacccgaccaaggtgaccatctttggcgagctggcgggcagcatgtcggtcatgtgccacattctctggaacgacggcgacaacacgtacaagggcaagccgctcttccgcgcgggcatcatgcagctgggggccatggtgccgctggacgccgtggacggcatctacggcaacgagatctttgacctcttggcgtcgaacgcgggctgcggcagcgccagcgacaagcttgcgtgcttgcgcggtgtgctgtacgacacgttggaggacgccaccaacaacacccctgggttcttggcgtactcctcgttgcggttgctgtacctcccccggcccgacggcgtgaacatcaccgacgacatgtacgccttggtgcgcgagggcaagtatgccaacatccctgtgatcatcggcgaccagaacgacgagggcaccttctttggcaccctgctgttgaacgtgaccacggatgcccaggcccgcgagtacttcaagcagctgtttgtccacgccagcgacgcggagatcgacacgttgatgacggcgtaccccggcgacatcacccagggcctgccgttcgacacgggtattctcaacgccctcaccccgcagttcaagagaatcctggcggtgctcggcgaccttggctttacgcttgctcgtcgctacttcctcaaccactacaccggcggcaccaagtactcattcctcctgaagcagctcctgggcttgccggtgctcggaacgttccactccaacgacattgtcttccaggactacttgttgggcagcggctcgctcatctacaacaacgcgttcattgcgtttgccacggacttggaccccaacaccgcggggttgttggtgaagtggcccgagtacaccagcagcctgcagctgggcaacaacttgatgatgatcaacgccttgggcttgtacaccggcaaggacaacttccgcaccgccggctacgacgcgttgttctccaacccgccgctgttctttgtgtga

SEQ ID NO: 13 - DNA, 1605 bp, synthetic construct
  misc_feature 1..1605: note = Mutant enzyme 6(S300P)
  source 1..1605: mol_type = other DNA
gcccccaccgccacgctcgccaacggcgacaccatcaccggtctcaacgccatcatcaacgaggcgttcctcggcattccctttgccgagccgccggtgggcaacctccgcttcaaggaccccgtgccgtactccggctcgctcgatggccagaagttcacgctgtacggcccgctgtgcatgcagcagaaccccgagggcacctacgaggagaacctccccaaggcagcgctcgacttggtgatgcagtccaaggtgtttgaggcggtgctgccgctgagcgaggactgtctcaccatcaacgtggtgcggccgccgggcaccaaggcgggtgccaacctcccggtgatgctctggatctttggcggcgggtttgaggtgggtggcaccagcaccttccctcccgcccagatgatcaccaagagcattgccatgggcaagcccatcatccacgtgagcgtcaactaccgcgtgtcgtcgtgggggttcttggctggcgacgagatcaaggccgagggcagtgccaacgccggtttgaaggaccagcgcttgggcatgcagtgggtggcggacaacattgcggcgtttggcggcgacccgaccaaggtgaccatctttggcgagctggcgggcagcatgtcggtcatgtgccacattctctggaacgacggcgacaacacgtacaagggcaagccgctcttccgcgcgggcatcatgcagctgggggccatggtgccgctggacgccgtggacggcatctacggcaacgagatctttgacctcttggcgtcgaacgcgggctgcggcagcgccagcgacaagcttgcgtgcttgcgcggtgtgctgagcgacacgttggaggacgccaccaacaacacccctgggttcttggcgtacccgtcgttgcggttgctgtacctcccccggcccgacggcgtgaacatcaccgacgacatgtacgccttggtgcgcgagggcaagtatgccaacatccctgtgatcatcggcgaccagaacgacgagggcaccttctttggcaccctgctgttgaacgtgaccacggatgcccaggcccgcgagtacttcaagcagctgtttgtccacgccagcgacgcggagatcgacacgttgatgacggcgtaccccggcgacatcacccagggcctgccgttcgacacgggtattctcaacgccctcaccccgcagttcaagagaatcctggcggtgctcggcgaccttggctttacgcttgctcgtcgctacttcctcaaccactacaccggcggcaccaagtactcattcctcctgaagcagctcctgggcttgccggtgctcggaacgttccactccaacgacattgtcttccaggactacttgttgggcagcggctcgctcatctacaacaacgcgttcattgcgtttgccacggacttggaccccaacaccgcggggttgttggtgaagtggcccgagtacaccagcagcctgcagctgggcaacaacttgatgatgatcaacgccttgggcttgtacaccggcaaggacaacttccgcaccgccggctacgacgcgttgttctccaacccgccgctgttctttgtgtga

SEQ ID NO: 14 - DNA, 1605 bp, synthetic construct
  misc_feature 1..1605: note = Mutant enzyme 1(T130C-S153C)
  source 1..1605: mol_type = other DNA
gcaccaactgcaaccttagcaaacggagacacaatcactggtttgaacgccattatcaacgaagccttcttgggaatcccatttgccgaaccacctgtcggaaacttgaggttcaaggacccagtaccttactcaggttcattggacggtcagaaattcacctcttacggtccatcttgtatgcaacagaatcctgagggaacctatgaggagaacttgccaaaagcagctttggatttggtcatgcagtcaaaagtcttcgaggccgtctcaccatcttctgaggactgtttgacaattaacgtcgttaggcctcctggaaccaaagccggtgctaatttgcctgtcatgttatggatcttcggaggaggttttgaagttggaggttgttctacatttccacctgcccagatgatcacaaaatctatcgccatgggaaagcctattatccacgtatgtgtcaactatagggtttcatcttggggttttttagctggagacgaaatcaaggctgaaggatcagcaaatgcaggtttaaaggaccagagattaggaatgcaatgggttgccgacaatatagcagcctttggtggagaccctacaaaggttaccattttcggagaatctgctggatctatgtcagtcatgtgccacatattgtggaacgatggagacaacacctacaagggtaaaccattgttcagagcaggtattatgcaatcaggtgccatggttccttctgatgctgttgacggtatctacggaaacgagattttcgacttattagcttctaacgccggatgcggatctgcctcagataagttggcatgtttaaggggagtctcttcagataccttggaggatgccaccaacaacacaccaggatttttggcctattcttctttgagattgtcatacttgcctagaccagacggagtcaatattactgacgacatgtacgcattagtcagagagggaaagtacgcaaacatcccagtcataattggagatcagaacgacgagggtacattcttcggtacctcatcattgaacgttacaacagatgctcaagcaagggagtatttcaaacaatcatttgttcacgcatctgacgccgaaatagacactttaatgaccgcctacccaggtgacataacccagggttcaccattcgatactggtatcttaaacgctttgacacctcagtttaaaaggatatcagctgttttgggtgacttaggattcacattagctagaagatacttcttgaatcactacactggtggtacaaagtattctttcttgtctaagcaattatcaggtttgccagttttaggaaccttccactctaatgacattgtcttccaagactacttgttgggatctggatcattaatctacaataacgcattcatcgcctttgccacagatttggaccctaacacagcaggattgttagtaaagtggcctgaatacacatcatcttcacagtctggaaacaatttgatgatgattaacgccttaggtttgtacaccggtaaagataactttaggacagctggttacgacgccttgttctctaacccaccttcatttttcgtatga

SEQ ID NO: 15 - DNA, 1605 bp, synthetic construct
  misc_feature 1..1605: note = Mutant enzyme 2(A249P)
  source 1..1605: mol_type = other DNA
gcaccaactgcaaccttagcaaacggagacacaatcactggtttgaacgccattatcaacgaagccttcttgggaatcccatttgccgaaccacctgtcggaaacttgaggttcaaggacccagtaccttactcaggttcattggacggtcagaaattcacctcttacggtccatcttgtatgcaacagaatcctgagggaacctatgaggagaacttgccaaaagcagctttggatttggtcatgcagtcaaaagtcttcgaggccgtctcaccatcttctgaggactgtttgacaattaacgtcgttaggcctcctggaaccaaagccggtgctaatttgcctgtcatgttatggatcttcggaggaggttttgaagttggaggtacatctacatttccacctgcccagatgatcacaaaatctatcgccatgggaaagcctattatccacgtatcagtcaactatagggtttcatcttggggttttttagctggagacgaaatcaaggctgaaggatcagcaaatgcaggtttaaaggaccagagattaggaatgcaatgggttgccgacaatatagcagcctttggtggagaccctacaaaggttaccattttcggagaatctgctggatctatgtcagtcatgtgccacatattgtggaacgatggagacaacacctacaagggtaaaccattgttcagagcaggtattatgcaatcaggtgccatggttccttctgatccggttgacggtatctacggaaacgagattttcgacttattagcttctaacgccggatgcggatctgcctcagataagttggcatgtttaaggggagtctcttcagataccttggaggatgccaccaacaacacaccaggatttttggcctattcttctttgagattgtcatacttgcctagaccagacggagtcaatattactgacgacatgtacgcattagtcagagagggaaagtacgcaaacatcccagtcataattggagatcagaacgacgagggtacattcttcggtacctcatcattgaacgttacaacagatgctcaagcaagggagtatttcaaacaatcatttgttcacgcatctgacgccgaaatagacactttaatgaccgcctacccaggtgacataacccagggttcaccattcgatactggtatcttaaacgctttgacacctcagtttaaaaggatatcagctgttttgggtgacttaggattcacattagctagaagatacttcttgaatcactacactggtggtacaaagtattctttcttgtctaagcaattatcaggtttgccagttttaggaaccttccactctaatgacattgtcttccaagactacttgttgggatctggatcattaatctacaataacgcattcatcgcctttgccacagatttggaccctaacacagcaggattgttagtaaagtggcctgaatacacatcatcttcacagtctggaaacaatttgatgatgattaacgccttaggtttgtacaccggtaaagataactttaggacagctggttacgacgccttgttctctaacccaccttcatttttcgtatga

SEQ ID NO: 16 - DNA, 1605 bp, synthetic construct
  misc_feature 1..1605: note = Mutant enzyme 3(F259Y)
  source 1..1605: mol_type = other DNA
gcaccaactgcaaccttagcaaacggagacacaatcactggtttgaacgccattatcaacgaagccttcttgggaatcccatttgccgaaccacctgtcggaaacttgaggttcaaggacccagtaccttactcaggttcattggacggtcagaaattcacctcttacggtccatcttgtatgcaacagaatcctgagggaacctatgaggagaacttgccaaaagcagctttggatttggtcatgcagtcaaaagtcttcgaggccgtctcaccatcttctgaggactgtttgacaattaacgtcgttaggcctcctggaaccaaagccggtgctaatttgcctgtcatgttatggatcttcggaggaggttttgaagttggaggtacatctacatttccacctgcccagatgatcacaaaatctatcgccatgggaaagcctattatccacgtatcagtcaactatagggtttcatcttggggttttttagctggagacgaaatcaaggctgaaggatcagcaaatgcaggtttaaaggaccagagattaggaatgcaatgggttgccgacaatatagcagcctttggtggagaccctacaaaggttaccattttcggagaatctgctggatctatgtcagtcatgtgccacatattgtggaacgatggagacaacacctacaagggtaaaccattgttcagagcaggtattatgcaatcaggtgccatggttccttctgatgctgttgacggtatctacggaaacgagatttacgacttattagcttctaacgccggatgcggatctgcctcagataagttggcatgtttaaggggagtctcttcagataccttggaggatgccaccaacaacacaccaggatttttggcctattcttctttgagattgtcatacttgcctagaccagacggagtcaatattactgacgacatgtacgcattagtcagagagggaaagtacgcaaacatcccagtcataattggagatcagaacgacgagggtacattcttcggtacctcatcattgaacgttacaacagatgctcaagcaagggagtatttcaaacaatcatttgttcacgcatctgacgccgaaatagacactttaatgaccgcctacccaggtgacataacccagggttcaccattcgatactggtatcttaaacgctttgacacctcagtttaaaaggatatcagctgttttgggtgacttaggattcacattagctagaagatacttcttgaatcactacactggtggtacaaagtattctttcttgtctaagcaattatcaggtttgccagttttaggaaccttccactctaatgacattgtcttccaagactacttgttgggatctggatcattaatctacaataacgcattcatcgcctttgccacagatttggaccctaacacagcaggattgttagtaaagtggcctgaatacacatcatcttcacagtctggaaacaatttgatgatgattaacgccttaggtttgtacaccggtaaagataactttaggacagctggttacgacgccttgttctctaacccaccttcatttttcgtatga

SEQ ID NO: 17 - DNA, 1605 bp, synthetic construct
  misc_feature 1..1605: note = Mutant enzyme 4(S282P)
  source 1..1605: mol_type = other DNA
gcaccaactgcaaccttagcaaacggagacacaatcactggtttgaacgccattatcaacgaagccttcttgggaatcccatttgccgaaccacctgtcggaaacttgaggttcaaggacccagtaccttactcaggttcattggacggtcagaaattcacctcttacggtccatcttgtatgcaacagaatcctgagggaacctatgaggagaacttgccaaaagcagctttggatttggtcatgcagtcaaaagtcttcgaggccgtctcaccatcttctgaggactgtttgacaattaacgtcgttaggcctcctggaaccaaagccggtgctaatttgcctgtcatgttatggatcttcggaggaggttttgaagttggaggtacatctacatttccacctgcccagatgatcacaaaatctatcgccatgggaaagcctattatccacgtatcagtcaactatagggtttcatcttggggttttttagctggagacgaaatcaaggctgaaggatcagcaaatgcaggtttaaaggaccagagattaggaatgcaatgggttgccgacaatatagcagcctttggtggagaccctacaaaggttaccattttcggagaatctgctggatctatgtcagtcatgtgccacatattgtggaacgatggagacaacacctacaagggtaaaccattgttcagagcaggtattatgcaatcaggtgccatggttccttctgatgctgttgacggtatctacggaaacgagattttcgacttattagcttctaacgccggatgcggatctgcctcagataagttggcatgtttaaggggagtcccgtcagataccttggaggatgccaccaacaacacaccaggatttttggcctattcttctttgagattgtcatacttgcctagaccagacggagtcaatattactgacgacatgtacgcattagtcagagagggaaagtacgcaaacatcccagtcataattggagatcagaacgacgagggtacattcttcggtacctcatcattgaacgttacaacagatgctcaagcaagggagtatttcaaacaatcatttgttcacgcatctgacgccgaaatagacactttaatgaccgcctacccaggtgacataacccagggttcaccattcgatactggtatcttaaacgctttgacacctcagtttaaaaggatatcagctgttttgggtgacttaggattcacattagctagaagatacttcttgaatcactacactggtggtacaaagtattctttcttgtctaagcaattatcaggtttgccagttttaggaaccttccactctaatgacattgtcttccaagactacttgttgggatctggatcattaatctacaataacgcattcatcgcctttgccacagatttggaccctaacacagcaggattgttagtaaagtggcctgaatacacatcatcttcacagtctggaaacaatttgatgatgattaacgccttaggtttgtacaccggtaaagataactttaggacagctggttacgacgccttgttctctaacccaccttcatttttcgtatga

SEQ ID NO: 18 - DNA, 1605 bp, synthetic construct
  misc_feature 1..1605: note = Mutant enzyme 5(S283Y)
  source 1..1605: mol_type = other DNA
gcaccaactgcaaccttagcaaacggagacacaatcactggtttgaacgccattatcaacgaagccttcttgggaatcccatttgccgaaccacctgtcggaaacttgaggttcaaggacccagtaccttactcaggttcattggacggtcagaaattcacctcttacggtccatcttgtatgcaacagaatcctgagggaacctatgaggagaacttgccaaaagcagctttggatttggtcatgcagtcaaaagtcttcgaggccgtctcaccatcttctgaggactgtttgacaattaacgtcgttaggcctcctggaaccaaagccggtgctaatttgcctgtcatgttatggatcttcggaggaggttttgaagttggaggtacatctacatttccacctgcccagatgatcacaaaatctatcgccatgggaaagcctattatccacgtatcagtcaactatagggtttcatcttggggttttttagctggagacgaaatcaaggctgaaggatcagcaaatgcaggtttaaaggaccagagattaggaatgcaatgggttgccgacaatatagcagcctttggtggagaccctacaaaggttaccattttcggagaatctgctggatctatgtcagtcatgtgccacatattgtggaacgatggagacaacacctacaagggtaaaccattgttcagagcaggtattatgcaatcaggtgccatggttccttctgatgctgttgacggtatctacggaaacgagattttcgacttattagcttctaacgccggatgcggatctgcctcagataagttggcatgtttaaggggagtctcttacgataccttggaggatgccaccaacaacacaccaggatttttggcctattcttctttgagattgtcatacttgcctagaccagacggagtcaatattactgacgacatgtacgcattagtcagagagggaaagtacgcaaacatcccagtcataattggagatcagaacgacgagggtacattcttcggtacctcatcattgaacgttacaacagatgctcaagcaagggagtatttcaaacaatcatttgttcacgcatctgacgccgaaatagacactttaatgaccgcctacccaggtgacataacccagggttcaccattcgatactggtatcttaaacgctttgacacctcagtttaaaaggatatcagctgttttgggtgacttaggattcacattagctagaagatacttcttgaatcactacactggtggtacaaagtattctttcttgtctaagcaattatcaggtttgccagttttaggaaccttccactctaatgacattgtcttccaagactacttgttgggatctggatcattaatctacaataacgcattcatcgcctttgccacagatttggaccctaacacagcaggattgttagtaaagtggcctgaatacacatcatcttcacagtctggaaacaatttgatgatgattaacgccttaggtttgtacaccggtaaagataactttaggacagctggttacgacgccttgttctctaacccaccttcatttttcgtatga

SEQ ID NO: 19 - DNA, 1605 bp, synthetic construct
  misc_feature 1..1605: note = Mutant enzyme 6(S300P)
  source 1..1605: mol_type = other DNA
gcaccaactgcaaccttagcaaacggagacacaatcactggtttgaacgccattatcaacgaagccttcttgggaatcccatttgccgaaccacctgtcggaaacttgaggttcaaggacccagtaccttactcaggttcattggacggtcagaaattcacctcttacggtccatcttgtatgcaacagaatcctgagggaacctatgaggagaacttgccaaaagcagctttggatttggtcatgcagtcaaaagtcttcgaggccgtctcaccatcttctgaggactgtttgacaattaacgtcgttaggcctcctggaaccaaagccggtgctaatttgcctgtcatgttatggatcttcggaggaggttttgaagttggaggtacatctacatttccacctgcccagatgatcacaaaatctatcgccatgggaaagcctattatccacgtatcagtcaactatagggtttcatcttggggttttttagctggagacgaaatcaaggctgaaggatcagcaaatgcaggtttaaaggaccagagattaggaatgcaatgggttgccgacaatatagcagcctttggtggagaccctacaaaggttaccattttcggagaatctgctggatctatgtcagtcatgtgccacatattgtggaacgatggagacaacacctacaagggtaaaccattgttcagagcaggtattatgcaatcaggtgccatggttccttctgatgctgttgacggtatctacggaaacgagattttcgacttattagcttctaacgccggatgcggatctgcctcagataagttggcatgtttaaggggagtctcttcagataccttggaggatgccaccaacaacacaccaggatttttggcctatccgtctttgagattgtcatacttgcctagaccagacggagtcaatattactgacgacatgtacgcattagtcagagagggaaagtacgcaaacatcccagtcataattggagatcagaacgacgagggtacattcttcggtacctcatcattgaacgttacaacagatgctcaagcaagggagtatttcaaacaatcatttgttcacgcatctgacgccgaaatagacactttaatgaccgcctacccaggtgacataacccagggttcaccattcgatactggtatcttaaacgctttgacacctcagtttaaaaggatatcagctgttttgggtgacttaggattcacattagctagaagatacttcttgaatcactacactggtggtacaaagtattctttcttgtctaagcaattatcaggtttgccagttttaggaaccttccactctaatgacattgtcttccaagactacttgttgggatctggatcattaatctacaataacgcattcatcgcctttgccacagatttggaccctaacacagcaggattgttagtaaagtggcctgaatacacatcatcttcacagtctggaaacaatttgatgatgattaacgccttaggtttgtacaccggtaaagataactttaggacagctggttacgacgccttgttctctaacccaccttcatttttcgtatga

SEQ ID NO: 20 - DNA, 45 bp, Candida cylindracea
  source 1..45: mol_type = other DNA
atggagctcgctcttgcgctcctgctcattgcctcggtggctgct

SEQ ID NO: 21 - protein, 15 aa, Candida cylindracea
MELALALSLIASVAA

SEQ ID NO: 22 - protein, 549 aa, Candida cylindracea
MELALALSLIASVAAAPTATLANGDTITGLNAIINEAFLGIPFAEPPVGNLRFKDPVPYSGSLDGQKFTSYGPSCMQQNPEGTYEENLPKAALDLVMQSKVFEAVSPSSEDCLTINVVRPPGTKAGANLPVMLWIFGGGFEVGGTSTFPPAQMITKSIAMGKPIIHVSVNYRVSSWGFLAGDEIKAEGSANAGLKDQRLGMQWVADNIAAFGGDPTKVTIFGESAGSMSVMCHILWNDGDNTYKGKPLFRAGIMQSGAMVPSDAVDGIYGNEIFDLLASNAGCGSASDKLACLRGVSSDTLEDATNNTPGFLAYSSLRLSYLPRPDGVNITDDMYALVREGKYANIPVIIGDQNDEGTFFGTSSLNVTTDAQAREYFKQSFVHASDAEIDTLMTAYPGDITQGSPFDTGILNALTPQFKRISAVLGDLGFTLARRYFLNHYTGGTKYSFLSKQLSGLPVLGTFHSNDIVFQDYLLGSGSLIYNNAFIAFATDLDPNTAGLLVKWPEYTSSSQSGNNLMMINALGLYTGKDNFRTAGYDALFSNPPSFFV

SEQ ID NO: 23 - DNA, 1650 bp, Candida cylindracea
  source 1..1650: mol_type = other DNA
atggagctcgctcttgcgctcctgctcattgcctcggtggctgctgcccccaccgccacgctcgccaacggcgacaccatcaccggtctcaacgccatcatcaacgaggcgttcctcggcattccctttgccgagccgccggtgggcaacctccgcttcaaggaccccgtgccgtactccggctcgctcgatggccagaagttcacgctgtacggcccgctgtgcatgcagcagaaccccgagggcacctacgaggagaacctccccaaggcagcgctcgacttggtgatgcagtccaaggtgtttgaggcggtgctgccgctgagcgaggactgtctcaccatcaacgtggtgcggccgccgggcaccaaggcgggtgccaacctcccggtgatgctctggatctttggcggcgggtttgaggtgggtggcaccagcaccttccctcccgcccagatgatcaccaagagcattgccatgggcaagcccatcatccacgtgagcgtcaactaccgcgtgtcgtcgtgggggttcttggctggcgacgagatcaaggccgagggcagtgccaacgccggtttgaaggaccagcgcttgggcatgcagtgggtggcggacaacattgcggcgtttggcggcgacccgaccaaggtgaccatctttggcgagctggcgggcagcatgtcggtcatgtgccacattctctggaacgacggcgacaacacgtacaagggcaagccgctcttccgcgcgggcatcatgcagctgggggccatggtgccgctggacgccgtggacggcatctacggcaacgagatctttgacctcttggcgtcgaacgcgggctgcggcagcgccagcgacaagcttgcgtgcttgcgcggtgtgctgagcgacacgttggaggacgccaccaacaacacccctgggttcttggcgtactcctcgttgcggttgctgtacctcccccggcccgacggcgtgaacatcaccgacgacatgtacgccttggtgcgcgagggcaagtatgccaacatccctgtgatcatcggcgaccagaacgacgagggcaccttctttggcaccctgctgttgaacgtgaccacggatgcccaggcccgcgagtacttcaagcagctgtttgtccacgccagcgacgcggagatcgacacgttgatgacggcgtaccccggcgacatcacccagggcctgccgttcgacacgggtattctcaacgccctcaccccgcagttcaagagaatcctggcggtgctcggcgaccttggctttacgcttgctcgtcgctacttcctcaaccactacaccggcggcaccaagtactcattcctcctgaagcagctcctgggcttgccggtgctcggaacgttccactccaacgacattgtcttccaggactacttgttgggcagcggctcgctcatctacaacaacgcgttcattgcgtttgccacggacttggaccccaacaccgcggggttgttggtgaagtggcccgagtacaccagcagcctgcagctgggcaacaacttgatgatgatcaacgccttgggcttgtacaccggcaaggacaacttccgcaccgccggctacgacgcgttgttctccaacccgccgctgttctttgtgtga

SEQ ID NO: 24 - protein, 534 aa, Candida cylindracea
APTATLANGDTITGLNAIVNEKFLGIPFAEPPVGTLRFKPPVPYSASLNGQQFTSYGPSCMQMNPMGSFEDTLPKNARHLVLQSKIFQVVLPNDEDCLTINVIRPPGTRASAGLPVMLWIFGGGFELGGSSLFPGDQMVAKSVLMGKPVIHVSMNYRVASWGFLAGPDIQNEGSGNAGLHDQRLAMQWVADNIAGFGGDPSKVTIYGESAGSMSTFVHLVWNDGDNTYNGKPLFRAAIMQSGCMVPSDPVDGTYGTEIYNQVVASAGCGSASDKLACLRGLSQDTLYQATSDTPGVLAYPSLRLSYLPRPDGTFITDDMYALVRDGKYAHVPVIIGDQNDEGTLFGLSSLNVTTDAQARAYFKQSFIHASDAEIDTLMAAYTSDITQGSPFDTGIFNAITPQFKRISALLGDLAFTLARRYFLNYYQGGTKYSFLSKQLSGLPVLGTFHGNDIIWQDYLVGSGSVIYNNAFIAFANDLDPNKAGLWTNWPTYTSSSQSGNNLMQINGLGLYTGKDNFRPDAYSALFSNPPSFFV

SEQ ID NO: 25 - protein, 534 aa, Candida cylindracea
APTAKLANGDTITGLNAIINEAFLGIPFAEPPVGNLRFKDPVPYSGSLNGQKFTSYGPSCMQQNPEGTFEENLGKTALDLVMQSKVFQAVLPQSEDCLTINVVRPPGTKAGANLPVMLWIFGGGFEIGSPTIFPPAQMVTKSVLMGKPIIHVAVNYRVASWGFLAGDDIKAEGSGNAGLKDQRLGMQWVADNIAGFGGDPSKVTIFGESAGSMSVLCHLIWNDGDNTYKGKPLFRAGIMQSGAMVPSDPVDGTYGNEIYDLFVSSAGCGSASDKLACLRSASSDTLLDATNNTPGFLAYSSLRLSYLPRPDGKNITDDMYKLVRDGKYASVPVIIGDQNDEGTIFGLSSLNVTTNAQARAYFKQSFIHASDAEIDTLMAAYPQDITQGSPFDTGIFNAITPQFKRISAVLGDLAFIHARRYFLNHFQGGTKYSFLSKQLSGLPIMGTFHANDIVWQDYLLGSGSVIYNNAFIAFATDLDPNTAGLLVNWPKYTSSSQSGNNLMMINALGLYTGKDNFRTAGYDALMTNPSSFFV

SEQ ID NO: 26 - protein, 534 aa, Candida cylindracea
APTATLANGDTITGLNAIINEAFLGIPFAQPPVGNLRFKPPVPYSASLNGQKFTSYGPSCMQMNPLGNWDSSLPKAAINSLMQSKLFQAVLPNGEDCLTINVVRPSGTKPGANLPVMVWIFGGGFEVGGSSLFPPAQMITASVLMGKPIIHVSMNYRVASWGFLAGPDIKAEGSGNAGLHDQRLGLQWVADNIAGFGGDPSKVTIFGESAGSMSVMCQLLWNDGDNTYNGKPLFRAAIMQSGAMVPSDPVDGPYGTQIYDQVVASAGCGSASDKLACLRSISNDKLFQATSDTPGALAYPSLRLSFLPRPDGTFITDDMFKLVRDGKCANVPVIIGDQNDEGTVFALSSLNVTTDAQARQYFKESFIHASDAEIDTLMAAYPSDITQGSPFDTGIFNAITPQFKRIAAVLGDLAFTLPRRYFLNHFQGGTKYSFLSKQLSGLPVIGTHHANDIVWQDFLVSHSSAVYNNAFIAFANDLDPNKAGLLVNWPKYTSSSQSGNNLLQINALGLYTGKDNFRTAGYDALFTNPSSFFV

SEQ ID NO: 27 - protein, 534 aa, Candida cylindracea
APTATLANGDTITGLNAIINEAFLGIPFAEPPVGNLRFKDPVPYRGSLNGQSFTAYGPSCMQQNPEGTYEENLPKVALDLVMQSKVFQAVLPNSEDCLTINVVRPPGTKAGANLPVMLWIFGGGFEIGSPTIFPPAQMVSKSVLMGKPIIHVAVNYRLASFGFLAGPDIKAEGSSNAGLKDQRLGMQWVADNIAGFGGDPSKVTIFGESAGSMSVLCHLLWNGGDNTYKGKPLFRAGIMQSGAMVPSDPVDGTYGTQIYDTLVASTGCSSASNKLACLRGLSTQALLDATNDTPGFLSYTSLRLSYLPRPDGANITDDMYKLVRDGKYASVPVIIGDQNDEGFLFGLSSLNTTTEADAEAYLRKSFIHATDADITALKAAYPSDVTQGSPFDTGILNALTPQLKRINAVLGDLTFTLSRRYFLNHYTGGPKYSFLSKQLSGLPILGTFHANDIVWQHFLLGSGSVIYNNAFIAFATDLDPNTAGLSVQWPKSTSSSQAGDNLMQISALGLYTGKDNFRTAGYNALFADPSHFFV

SEQ ID NO: 28 - protein, 549 aa, Diutina rugosa
MELALALSLIASVAAAPTATLANGDTITGLNAIINEAFLGIPFAEPPVGNLRFKDPVPYRGSLNGQSFTAYGPSCMQQNPEGTYEENLPKVALDLVMQSKVFQAVLSNSEDCLTINVVRPPGTKAGANLPVMLWIFGGGFEIGSPTIFPPAQMVSKSVLMGKPIIHVAVNYRLASFGFLAGPDIKAEGSSNAGLKDQRLGMQWVADNIAGFGGDPSKVTIFGESAGSMSVLCHLLWNGGDNTYKGKPLFRAGIMQSGAMVPSDPVDGTYGTQIYDTLVASTGCSSASNKLACLRGLSTQALLDATNDTPGFLAFSSLRLSYLPRPDGVNITDDFYALVRNGKYAHVPVIIGDQNDEGTIFGLSSLNVTTNAQAREYFKQSFIHASDAEIDTLMTAYPQDITQGSPFDTGVLNALTPQFKRISAVLGDLAFTLARRYFLNYYQGGTKYSFLSKQLSGLPVLGTFHSNDLTFQNDLLGSGSLIYDNAFIAFVNDLDPNKAGLLVNWPTYTSSSQSGNNMMMINALGLYTGKDNFRTAGYDALFANPPSFFV

SEQ ID NO: 29 - protein, 549 aa, Candida cylindracea
MKLALALLLIASVAAAPTAKLANGDTITGLNAIINEAFLGIPFAEPPVGNLRFKDPVPYSGSLNGQKFTLYGPLCMQQNPEGTFEENLGKTALDLVMQSKVFQAVLPQSEDCLTINVVRPPGTKAGANLPVMLWIFGGGFEIGSPTIFPPAQMVTKSVLMGKPIIHVAVNYRVASWGFLAGDDIKAEGSGNAGLKDQRLGMQWVADNIAGFGGDPSKVTIFGELAGSMSVLCHLIWNDGDNTYKGKPLFRAGIMQLGAMVPLDPVDGTYGNEIYDLFVSSAGCGSASDKLACLRSALSDTLLDATNNTPGFLAYSSLRLLYLPRPDGKNITDDMYKLVRDGKYASVPVIIGDQNDEGTIFGLLLLNVTTNAQARAYFKQLFIHASDAEIDTLMAAYPQDITQGLPFDTGIFNAITPQFKRILAVLGDLAFIHARRYFLNHFQGGTKYSFLLKQLLGLPIMGTFHANDIVWQDYLLGSGSVIYNNAFIAFATDLDPNTAGLLVNWPKYTSSLQLGNNLMMINALGLYTGKDNFRTAGYDALMTNPLLFFV

SEQ ID NO: 30 - protein, 534 aa, Candida sp. AC-IITM
APTATLANGDTITGVNKIVNEAFLGIPFAEPPVGNLRFKDPVPYSRSLNGQKFTLNGPLCMQMNPLGNWDSSLPKAAINLLMQSKLFQAVLPNGEDCLTINVVRPLGTKPGANLPVMVWIFGGGFEVGGSSLFPPAQMITASVLMGKPIIHVSMNYRVASWGFLAGPDIKAEGSGNAGLHDQRLGLQWVADNIAGFGGDPSKVTIFGELAGSMSVMCQLLWNDGDNTYNGKPLFRAAIMQLGAMVPLDPVDGPYGTQIYDQVVASAGCGSASDKLACLRSILNDKLFQATSDTPGALAYPSLRLLFLPRPDGTFITDDMFKLVRDGKCANIPVIIGDQNDEGTFFGTLLLNVTTDAQAREYFKQLFVHASDAEIDTLMTAYPGDITQGLPFDTGILNALTPQFKRILAVLGDLGFTLARRYFLNHYTGGTKYSFLLKQLLGLPVLGTFHSNDIVFQDYLLGSGSLIYNNAFIAFATDLDPNTAGLLVKWPEYTSSLQLGNNLMMINALGLYTGKDNFRTAGYDALFSNPLLFFV